European Patent Application EP 4 806 461 A1, published September 16, 2026. Title: ROUGH ATTENUATED BRUCELLA STRAIN, USE, VACCINE, ANTIGEN, AND KIT THEREOF. Applicant: INSTITUTE OF ANIMAL SCIENCES OF CHINESE ACADEMY OF AGRICULTURAL SCIENCES. Application EP. The sequence listing filed with the application follows.

SEQUENCE LISTING (4 sequences)

SEQ ID NO: 1 - DNA, 23 bp, synthetic construct
  source 1..23: mol_type = other DNA
gcgcggttttctgaaggttcagg

SEQ ID NO: 2 - DNA, 22 bp, synthetic construct
  source 1..22: mol_type = other DNA
aaatcgcgtccttgctggtctg

SEQ ID NO: 3 - DNA, 24 bp, synthetic construct
  source 1..24: mol_type = other DNA
gacgaacggaatttttccaatccc

SEQ ID NO: 4 - DNA, 24 bp, synthetic construct
  source 1..24: mol_type = other DNA
tgccgatcacttaagggccttcat